European Patent Specification EP 3 414 373 B1, published April 24, 2024. Title: COMPOSITE MATERIALS COMPRISING SYNTHETIC DRAGLINE SPIDER SILK. Applicant: SEEVIX MATERIAL SCIENCES LTD. The sequence listing filed with the application follows.

SEQUENCE LISTING (17 sequences)

SEQ ID NO: 1 - protein, 28 aa, artificial
  synthetic
  MISC_FEATURE (1)..(1): X is A or G
  MISC_FEATURE (2)..(2): X is S or G
  MISC_FEATURE (10)..(10): X is G or E
  MISC_FEATURE (11)..(11): X is G, S or N
  MISC_FEATURE (12)..(12): X is Q or Y
  MISC_FEATURE (15)..(15): X is G or S
  MISC_FEATURE (17)..(17): X is P or R
  MISC_FEATURE (20)..(20): X is Y or Q
  MISC_FEATURE (27)..(27): X is G or S
  MISC_FEATURE (28)..(28): X is S or G
XXGPGGYGPXXXGPXGXGGXGPGGPGXX

SEQ ID NO: 2 - protein, 27 aa, artificial
  synthetic
SGPGGYGPGSQGPSGPGGYGPGGPGSS

SEQ ID NO: 3 - protein, 35 aa, artificial
  synthetic
AAAAAAAASGPGGYGPGSQGPSGPGGYGPGGPGSS

SEQ ID NO: 4 - protein, 35 aa, artificial
  synthetic
AAAAAAAASGPGGYGPENQGPSGPGGYGPGGPGSS

SEQ ID NO: 5 - protein, 40 aa, artificial
  synthetic
MSYYHHHHHHDYDIPTTENLYFQGAMDPEFKGLRRRAQLV

SEQ ID NO: 6 - protein, 50 aa, artificial
  synthetic
MSYYHHHHHHDYDIPTTENLYFQGAMDPEFKGLRRRAQLVRPLSNLDNAP

SEQ ID NO: 7 - protein, 54 aa, artificial
  synthetic
MSYYHHHHHHDYDIPTTENLYFQGAMDPEFKGLRRRAQLVDPPGCRNSARAGSS

SEQ ID NO: 8 - protein, 97 aa, artificial
  synthetic
  MISC_FEATURE (1)..(1): X is A or G
  MISC_FEATURE (2)..(2): X is S or G
  MISC_FEATURE (11)..(11): X is S or G
  MISC_FEATURE (12)..(12): X is Q or Y
  MISC_FEATURE (15)..(15): X is S or G
  MISC_FEATURE (17)..(17): X is P or R
  MISC_FEATURE (20)..(20): X is Y or Q
  MISC_FEATURE (27)..(27): X is G or S
  MISC_FEATURE (28)..(28): X is G or S
VAASRLSSPAASSRVSSAVSSLVSSGPTNGAAVSGALNSLVSQISASNPGLSGCDALVQALLELVSALVAILSSASIGQVNVSSVSQSTQMISQALS

SEQ ID NO: 9 - protein, 114 aa, artificial
  synthetic
GPSGPGAYGPSPSASASVAASRLSSPAASSRVSSAVSSLVSSGPTNGAAVSGALNSLVSQISASNPGLSGCDALVQALLELVSALVAILSSASIGQVNVSSVSQSTQMISQALS

SEQ ID NO: 10 - protein, 555 aa, artificial
  synthetic
AAAAAAASGSGGYGPENQGPSGPVAYGPGGPVSSAAAAAAAGSGPGGYGPENQGPSGPGGYGPGGSGSSAAAAAAAASGPGGYGPGSQGPSGPGGSGGYGPGSQGPSGPGASSAAAAAAAASGPGGYGPGSQGPSGPGAYGPGGPGSSAAASGPGGYGPGSQGPSGPGGSGGYGPGSQGPSGPGGPGASAAAAAAAAASGPGGYGPGSQGPSGPGAYGPGGPGSSAAASGPGGYGPGSQGPSGPGAYGPGGPGSSAAAAAAAGSGPGGYGPGNQGPSGPGGYGPGGPGSSAAAAAAASGPGGYGPGSQGPSGPGVYGPGGPGSSAAAAAAAGSGPGGYGPGNQGPSGPGGYGPGGSGSSAAAAAAAASGPGGYGPGSQGPSGPGGSGGYGPGSQGPSGPGASSAAAAAAAASGPGGYGPGSQGPSGPGAYGPGGPGSSAAASGPGGYGPGSQGPSGPGAYGPGGPGSSAAAAAAASGPGGYGPGSQGPSGPGGSRGYGPGSQGPGGPGASAAAAAAAAASGPGGYGPGSQGPSGPGYQGPSGPGAYGPSPSASAS

SEQ ID NO: 11 - protein, 6 aa, artificial
  synthetic
HHHHHH

SEQ ID NO: 12 - protein, 9 aa, artificial
  synthetic
YPYDVPDYA

SEQ ID NO: 13 - protein, 11 aa, artificial
  synthetic
MASMTGGQQMG

SEQ ID NO: 14 - protein, 35 aa, artificial
  synthetic
SGPGGYGPGSQGPSGPGGYGPGGPGSSAAAAAAAA

SEQ ID NO: 15 - DNA, 105 bp, Artificial
  Synthetic
tctggtcctggaggttatggcccaggaagccaaggaccatctggtccaggaggatatggtccaggcggacctggctctagtgcagcagctgccgcagcagctgca

SEQ ID NO: 16 - DNA, 28 bp, Artificial
  Synthetic
atatgctgcaggccctagtggtcctgga

SEQ ID NO: 17 - DNA, 20 bp, Artificial
  Synthetic
tcgacaagcttggtaccgca